European Patent Application EP 4 678 744 A1, published January 14, 2026. Title: 아데닌 염기 교정 시스템. Applicant: 주식회사 그린진. Application KR. The sequence listing filed with the application follows.

SEQUENCE LISTING (18 sequences)

SEQ ID NO: 1 - protein, 166 aa, Artificial
SEVEFSHEYWMRHALTLAKRARDEREVPVGAVLVLNNRVIGEGWNRAIGLHDPTAHAEIMALRQGGLVMQNYRLIDATLYVTFEPCVMCAGAMIHSRIGRVVFGVRNSKRGAAGSLMNVLNYPGMNHRVEITEGILADECAALLCDFYRMPRQVFNAQKKAQSSIN

SEQ ID NO: 2 - protein, 138 aa, Burkholderia cenocepacia
GSYALGPYQISAPQLPAYNGQTVGTFYYVNDAGGLESKVFSSGGPTPYPNYANAGHVEGQSALFMRDNGISEGLVFHNNPEGTCGFCVNMTETLLPENAKMTVVPPEGAIPVKRGATGETKVFTGNSNSPKSPTKGGC

SEQ ID NO: 3 - protein, 44 aa, Artificial
GSYALGPYQISAPQLPAYNGQTVGTFYYVNDAGGLESKVFSSGG

SEQ ID NO: 4 - protein, 94 aa, Artificial
PTPYPNYANAGHVEGQSALFMRDNGISEGLVFHNNPEGTCGFCVNMTETLLPENAKMTVVPPEGAIPVKRGATGETKVFTGNSNSPKSPTKGGC

SEQ ID NO: 5 - protein, 108 aa, Artificial
GSYALGPYQISAPQLPAYNGQTVGTFYYVNDAGGLESKVFSSGGPTPYPNYANAGHVEGQSALFMRDNGISEGLVFHNNPEGTCGFCVNMTETLLPENAKMTVVPPEG

SEQ ID NO: 6 - protein, 30 aa, Artificial
AIPVKRGATGETKVFTGNSNSPKSPTKGGC

SEQ ID NO: 7 - protein, 330 aa, Artificial [sequence omitted]

SEQ ID NO: 8 - protein, 54 aa, Artificial
MDSQLVLSLKLNPSFTPLSPLFPFTPCSSFSPSLRFSSCYSRRLYSPVTVYAAK

SEQ ID NO: 9 - protein, 138 aa, Artificial
GSYALGPYQISAPQLPAYNGQTVGTFYYVNDAGGLEGKVFSSGGPTPYPNYANAGHVESQSALFMRDNGISEGLVFHNNPEGTCGFCVNMTETLLPENAKMTVVPPEGVIPVKRGATGETKVFTGNSNGPKSPTKGGC

SEQ ID NO: 10 - protein, 808 aa, Artificial
DLRTLGYSQQQQEKIKPKVRSTVAQHHEALVGHGFTHAHIVALSQHPAALGTVAVKYQDMIAALPEATHEAIVGVGKQWSGARALEALLTVAGELRGPPLQLDTGQLLKIAKRGGVTAVEAVHAWRNALTGAPLNLTPAQVVAIASHDGGKQALETVQRLLPVLCQAHGLTPAQVVAIASNGGGKQALETVQRLLPVLCQDHGLTPDQVVAIASNNGGKQALETVQRLLPVLCQDHGLTPAQVVAIASNNGGKQALETVQRLLPVLCQDHGLTPEQVVAIASNGGGKQALETVQRLLPVLCQAHGLTPAQVVAIASNGGGKQALETVQRLLPVLCQDHGLTPAQVVAIASHDGGKQALETVQRLLPVLCQDHGLTPDQVVAIASHDGGKQALETVQRLLPVLCQAHGLTPEQVVAIASNNGGKQALETVQRLLPVLCQAHGLTPAQVVAIASNNGGKQALETVQRLLPVLCQAHGLTPDQVVAIASHDGGKQALETVQRLLPVLCQDHGLTPAQVVAIASNNGGKQALETVQRLLPVLCQAHGLTPDQVVAIASNIGGKQALETVQRLLPVLCQAHGLTPDQVVAIASNIGGKQALETVQRLLPVLCQAHGLTPAQVVAIASHDGGKQALETVQRLLPVLCQAHGLTPEQVVAIASNNGGKQALETVQRLLPVLCQAHGLTPDQVVAIASNIGGKQALETVQRLLPVLCQDHGLTPDQVVAIASNIGGKQALETVQRLLPVLCQAHGLTPEQVVAIASNGGGKQALESIVAQLSRPDPALAALTNDHLVALACLGGRPALDAVKKGLG

SEQ ID NO: 11 - protein, 808 aa, Artificial
DLRTLGYSQQQQEKIKPKVRSTVAQHHEALVGHGFTHAHIVALSQHPAALGTVAVKYQDMIAALPEATHEAIVGVGKQWSGARALEALLTVAGELRGPPLQLDTGQLLKIAKRGGVTAVEAVHAWRNALTGAPLNLTPEQVVAIASNNGGKQALETVQRLLPVLCQAHGLTPDQVVAIASNGGGKQALETVQRLLPVLCQDHGLTPAQVVAIASNNGGKQALETVQRLLPVLCQAHGLTPEQVVAIASNGGGKQALETVQRLLPVLCQAHGLTPAQVVAIASNGGGKQALETVQRLLPVLCQAHGLTPDQVVAIASNNGGKQALETVQRLLPVLCQDHGLTPAQVVAIASNGGGKQALETVQRLLPVLCQDHGLTPAQVVAIASHDGGKQALETVQRLLPVLCQAHGLTPEQVVAIASHDGGKQALETVQRLLPVLCQAHGLTPAQVVAIASNNGGKQALETVQRLLPVLCQAHGLTPDQVVAIASNNGGKQALETVQRLLPVLCQDHGLTPAQVVAIASNIGGKQALETVQRLLPVLCQAHGLTPAQVVAIASNIGGKQALETVQRLLPVLCQDHGLTPDQVVAIASNIGGKQALETVQRLLPVLCQDHGLTPDQVVAIASNNGGKQALETVQRLLPVLCQAHGLTPAQVVAIASNIGGKQALETVQRLLPVLCQAHGLTPAQVVAIASNNGGKQALETVQRLLPVLCQDHGLTPAQVVAIASNNGGKQALETVQRLLPVLCQAHGLTPEQVVAIASNGGGKQALESIVAQLSRPDPALAALTNDHLVALACLGGRPALDAVKKGLG

SEQ ID NO: 12 - protein, 16 aa, Artificial
SGSETPGTSESATPES

SEQ ID NO: 13 - protein, 18 aa, Artificial
GSSGSETPGTSESATPES

SEQ ID NO: 14 - protein, 808 aa, Artificial
DLRTLGYSQQQQEKIKPKVRSTVAQHHEALVGHGFTHAHIVALSQHPAALGTVAVKYQDMIAALPEATHEAIVGVGKQWSGARALEALLTVAGELRGPPLQLDTGQLLKIAKRGGVTAVEAVHAWRNALTGAPLNLTPDQVVAIASNGGGKQALETVQRLLPVLCQAHGLTPAQVVAIASNGGGKQALETVQRLLPVLCQAHGLTPEQVVAIASNGGGKQALETVQRLLPVLCQAHGLTPEQVVAIASNNGGKQALETVQRLLPVLCQAHGLTPAQVVAIASNNGGKQALETVQRLLPVLCQDHGLTPDQVVAIASHDGGKQALETVQRLLPVLCQDHGLTPEQVVAIASHDGGKQALETVQRLLPVLCQAHGLTPAQVVAIASNNGGKQALETVQRLLPVLCQAHGLTPAQVVAIASNIGGKQALETVQRLLPVLCQAHGLTPEQVVAIASNGGGKQALETVQRLLPVLCQAHGLTPAQVVAIASNGGGKQALETVQRLLPVLCQAHGLTPDQVVAIASNNGGKQALETVQRLLPVLCQDHGLTPAQVVAIASNIGGKQALETVQRLLPVLCQAHGLTPDQVVAIASNGGGKQALETVQRLLPVLCQAHGLTPDQVVAIASNGGGKQALETVQRLLPVLCQAHGLTPDQVVAIASNGGGKQALETVQRLLPVLCQDHGLTPEQVVAIASNGGGKQALETVQRLLPVLCQAHGLTPDQVVAIASHDGGKQALETVQRLLPVLCQAHGLTPEQVVAIASNGGGKQALESIVAQLSRPDPALAALTNDHLVALACLGGRPALDAVKKGLG

SEQ ID NO: 15 - protein, 808 aa, Artificial
DLRTLGYSQQQQEKIKPKVRSTVAQHHEALVGHGFTHAHIVALSQHPAALGTVAVKYQDMIAALPEATHEAIVGVGKQWSGARALEALLTVAGELRGPPLQLDTGQLLKIAKRGGVTAVEAVHAWRNALTGAPLNLTPEQVVAIASNNGGKQALETVQRLLPVLCQAHGLTPAQVVAIASNNGGKQALETVQRLLPVLCQDHGLTPDQVVAIASHDGGKQALETVQRLLPVLCQDHGLTPEQVVAIASHDGGKQALETVQRLLPVLCQAHGLTPAQVVAIASNNGGKQALETVQRLLPVLCQAHGLTPAQVVAIASNIGGKQALETVQRLLPVLCQDHGLTPEQVVAIASNGGGKQALETVQRLLPVLCQAHGLTPAQVVAIASNGGGKQALETVQRLLPVLCQAHGLTPDQVVAIASNNGGKQALETVQRLLPVLCQAHGLTPAQVVAIASNIGGKQALETVQRLLPVLCQAHGLTPDQVVAIASNGGGKQALETVQRLLPVLCQAHGLTPDQVVAIASNGGGKQALETVQRLLPVLCQAHGLTPDQVVAIASNGGGKQALETVQRLLPVLCQDHGLTPEQVVAIASNGGGKQALETVQRLLPVLCQAHGLTPDQVVAIASHDGGKQALETVQRLLPVLCQAHGLTPAQVVAIASHDGGKQALETVQRLLPVLCQDHGLTPEQVVAIASNIGGKQALETVQRLLPVLCQAHGLTPAQVVAIASNIGGKQALETVQRLLPVLCQDHGLTPEQVVAIASNGGGKQALESIVAQLSRPDPALAALTNDHLVALACLGGRPALDAVKKGLG

SEQ ID NO: 16 - protein, 808 aa, Artificial
DLRTLGYSQQQQEKIKPKVRSTVAQHHEALVGHGFTHAHIVALSQHPAALGTVAVKYQDMIAALPEATHEAIVGVGKQWSGARALEALLTVAGELRGPPLQLDTGQLLKIAKRGGVTAVEAVHAWRNALTGAPLNLTPDQVVAIASNNGGKQALETVQRLLPVLCQAHGLTPAQVVAIASNGGGKQALETVQRLLPVLCQDHGLTPAQVVAIASNIGGKQALETVQRLLPVLCQAHGLTPAQVVAIASNIGGKQALETVQRLLPVLCQDHGLTPDQVVAIASNIGGKQALETVQRLLPVLCQDHGLTPDQVVAIASNNGGKQALETVQRLLPVLCQAHGLTPDQVVAIASNIGGKQALETVQRLLPVLCQAHGLTPDQVVAIASNIGGKQALETVQRLLPVLCQAHGLTPAQVVAIASHDGGKQALETVQRLLPVLCQAHGLTPDQVVAIASNNGGKQALETVQRLLPVLCQDHGLTPAQVVAIASNIGGKQALETVQRLLPVLCQAHGLTPEQVVAIASNNGGKQALETVQRLLPVLCQAHGLTPDQVVAIASNIGGKQALETVQRLLPVLCQAHGLTPDQVVAIASNIGGKQALETVQRLLPVLCQDHGLTPDQVVAIASNGGGKQALETVQRLLPVLCQAHGLTPAQVVAIASNGGGKQALETVQRLLPVLCQAHGLTPDQVVAIASNNGGKQALETVQRLLPVLCQAHGLTPAQVVAIASNGGGKQALETVQRLLPVLCQDHGLTPEQVVAIASNGGGKQALESIVAQLSRPDPALAALTNDHLVALACLGGRPALDAVKKGLG

SEQ ID NO: 17 - protein, 774 aa, Artificial
DLRTLGYSQQQQEKIKPKVRSTVAQHHEALVGHGFTHAHIVALSQHPAALGTVAVKYQDMIAALPEATHEAIVGVGKQWSGARALEALLTVAGELRGPPLQLDTGQLLKIAKRGGVTAVEAVHAWRNALTGAPLNLTPDQVVAIASNNGGKQALETVQRLLPVLCQAHGLTPAQVVAIASNGGGKQALETVQRLLPVLCQDHGLTPAQVVAIASNIGGKQALETVQRLLPVLCQAHGLTPAQVVAIASNIGGKQALETVQRLLPVLCQDHGLTPDQVVAIASNIGGKQALETVQRLLPVLCQDHGLTPDQVVAIASNNGGKQALETVQRLLPVLCQAHGLTPDQVVAIASNIGGKQALETVQRLLPVLCQAHGLTPDQVVAIASNIGGKQALETVQRLLPVLCQAHGLTPAQVVAIASHDGGKQALETVQRLLPVLCQAHGLTPDQVVAIASNNGGKQALETVQRLLPVLCQDHGLTPAQVVAIASNIGGKQALETVQRLLPVLCQAHGLTPEQVVAIASNNGGKQALETVQRLLPVLCQAHGLTPDQVVAIASNIGGKQALETVQRLLPVLCQAHGLTPDQVVAIASNIGGKQALETVQRLLPVLCQDHGLTPDQVVAIASNGGGKQALETVQRLLPVLCQAHGLTPEQVVAIASNGGGKQALETVQRLLPVLCQAHGLTPAQVVAIASNNGGKQALETVQRLLPVLCQDHGLTPEQVVAIASNGGGKQALESIVAQLSRPDPALAALTNDHLVALACLGGRPALDAVKKGLG

SEQ ID NO: 18 - protein, 16 aa, Artificial
SGSETPGTSESATPES